European Patent Application EP 4 339 208 A1, published March 20, 2024. Title: Anti-TIGIT antibodies and use thereof. Applicant: MediMabBio Inc. The sequence listing filed with the application follows.

SEQUENCE LISTING (31 sequences)

SEQ ID NO: 1 - protein, 6 aa, Artificial Sequence
  Synthetic_CDR-H1
SDYAWN

SEQ ID NO: 2 - protein, 16 aa, Artificial Sequence
  Synthetic_CDR-H2
YISYSGSARYNPSLKS

SEQ ID NO: 3 - protein, 9 aa, Artificial Sequence
  Synthetic_CDR-H3
KGYPAYFAY

SEQ ID NO: 4 - protein, 11 aa, Artificial Sequence
  Synthetic_CDR-L1, wherein X is K or R
XASQDVSTAVA

SEQ ID NO: 5 - protein, 7 aa, Artificial Sequence
  Synthetic_CDR-L2
SASYRYT

SEQ ID NO: 6 - protein, 9 aa, Artificial Sequence
  Synthetic_CDR-L3
QHHYSTPYT

SEQ ID NO: 7 - protein, 11 aa, Artificial Sequence
  Synthetic_CDR-L1
KASQDVSTAVA

SEQ ID NO: 8 - protein, 11 aa, Artificial Sequence
  Synthetic_CDR-L1
RASQDVSTAVA

SEQ ID NO: 9 - protein, 118 aa, Artificial Sequence
  Synthetic_Heavy chain variable region
DVQLQESGPGLVKPSQSLSLTCTVTGYSITSDYAWNWIRQFPGNKLEWMGYISYSGSARYNPSLKSRISITRDTSMNQFFLQLNSVTAEDTATYYCARKGYPAYFAYWGQGTLVTVSS

SEQ ID NO: 10 - protein, 118 aa, Artificial Sequence
  Synthetic_Heavy chain variable region
DVQLQESGPGLVKPSQTLSLTCTVTGYSITSDYAWNWIRQPPGKGLEWMGYISYSGSARYNPSLKSRITISRDTSMNQFSLKLNSVTAEDTATYYCARKGYPAYFAYWGQGTLVTVSS

SEQ ID NO: 11 - protein, 118 aa, Artificial Sequence
  Synthetic_Heavy chain variable region
DVQLQESGPGLVKPSQTLSLTCTVTGYSITSDYAWNWIRQPPGKGLEWMGYISYSGSARYNPSLKSRITISRDTSKNQFSLKLSSVTAEDTATYYCARKGYPAYFAYWGQGTLVTVSS

SEQ ID NO: 12 - protein, 118 aa, Artificial Sequence
  Synthetic_Heavy chain variable region
QVQLQESGPGLVKPSQTLSLTCTVTGYSITSDYAWNWIRQPPGKGLEWMGYISYSGSARYNPSLKSRVTISRDTSKNQFSLKLSSVTAEDTATYYCARKGYPAYFAYWGQGTLVTVSS

SEQ ID NO: 13 - protein, 118 aa, Artificial Sequence
  Synthetic_Heavy chain variable region
QVQLQESGPGLVKPSQTLSLTCTVTGYSITSDYAWNWIRQPPGKGLEWMGYISYSGSARYNPSLKSRVTISRDTSKNQFSLKLSSVTAADTAVYYCARKGYPAYFAYWGQGTLVTVSS

SEQ ID NO: 14 - protein, 118 aa, Artificial Sequence
  Synthetic_Heavy chain variable region
QVQLQESGPGLVKPSQTLSLTCTVTGYSITSDYAWNWIRQPPGKGLEWMGYISYSGSARYNPSLKSRVTISVDTSKNQFSLKLSSVTAADTAVYYCARKGYPAYFAYWGQGTLVTVSS

SEQ ID NO: 15 - protein, 107 aa, Artificial Sequence
  Synthetic_Light chain variable region
DIVMTQSHKFMSTSVGDRVSISCKASQDVSTAVAWYQQKPGQSPELLIYSASYRYTGVPDRFTGSGSGTDFTFTISSVQAEDLAVYYCQHHYSTPYTFGGGTKLEMK

SEQ ID NO: 16 - protein, 107 aa, Artificial Sequence
  Synthetic_Light chain variable region
DIVMTQSHSFLSASVGDRVSITCKASQDVSTAVAWYQQKPGQAPELLIYSASYRYTGVPDRFTGSGSGTDFTLTISSLQAEDVAVYYCQHHYSTPYTFGQGTKLEMK

SEQ ID NO: 17 - protein, 107 aa, Artificial Sequence
  Synthetic_Light chain variable region
DIVMTQSPSSLSASVGDRVSITCKASQDVSTAVAWYQQKPGQAPRLLIYSASYRYTGVPDRFTGSGSGTDFTLTISSLQAEDVAVYYCQHHYSTPYTFGQGTKLEIK

SEQ ID NO: 18 - protein, 107 aa, Artificial Sequence
  Synthetic_Light chain variable region
DIQMTQSPSSLSASVGDRVSITCKASQDVSTAVAWYQQKPGQAPRLLIYSASYRYTGVPDRFSGSGSGTDFTLTISSLQAEDVAVYYCQHHYSTPYTFGQGTKLEIK

SEQ ID NO: 19 - protein, 107 aa, Artificial Sequence
  Synthetic_Light chain variable region
DIQMTQSPSSLSASVGDRVTITCRASQDVSTAVAWYQQKPGQAPRLLIYSASYRYTGVPDRFSGSGSGTDFTLTISSLQAEDVAVYYCQHHYSTPYTFGQGTKLEIK

SEQ ID NO: 20 - protein, 107 aa, Artificial Sequence
  Synthetic_Light chain variable region
DIQMTQSPSSLSASVGDRVSITCKASQDVSTAVAWYQQKPGQAPRLLIYSASYRYTGVPDRFSGSGSGTDFTLTISSLQPEDFATYYCQHHYSTPYTFGQGTKLEIK

SEQ ID NO: 21 - protein, 330 aa, Artificial Sequence
  Synthetic_Heavy chain constant region
ASTKGPSVFPLAPSSKSTSGGTAALGCLVKDYFPEPVTVSWNSGALTSGVHTFPAVLQSSGLYSLSSVVTVPSSSLGTQTYICNVNHKPSNTKVDKRVEPKSCDKTHTCPPCPAPELLGGPSVFLFPPKPKDTLMISRTPEVTCVVVDVSHEDPEVKFNWYVDGVEVHNAKTKPREEQYNSTYRVVSVLTVLHQDWLNGKEYKCKVSNKALPAPIEKTISKAKGQPREPQVYTLPPSREEMTKNQVSLTCLVKGFYPSDIAVEWESNGQPENNYKTTPPVLDSDGSFFLYSKLTVDKSRWQQGNVFSCSVMHEALHNHYTQKSLSLSPGK

SEQ ID NO: 22 - protein, 107 aa, Artificial Sequence [sequence omitted]

SEQ ID NO: 23 - DNA, 354 bp, Artificial Sequence
  Synthetic_7A6 heavy chain variable region coding DNA
gatgtgcagcttcaggagtcgggacctggcctggtgaaaccttctcagtctctgtccctcacctgcactgtcactggctactcaatcaccagtgattatgcctggaactggatccggcagtttccaggaaacaaactggagtggatgggctacataagctacagtggtagcgctcgctacaacccatctctcaaaagtcgaatctctatcactcgagacacatccatgaaccagttcttcctgcagttgaattctgtgactgctgaggacacagccacatattactgtgcaagaaaggggtaccctgcctactttgcttactggggccaagggactctggtcactgtctctgca

SEQ ID NO: 24 - DNA, 321 bp, Artificial Sequence
  Synthetic_7A6 light chain variable region coding DNA
gacattgtgatgacccagtctcacaaattcatgtccacatcagtaggagacagggtcagcatctcctgcaaggccagtcaggatgtgagtactgctgtagcctggtatcaacagaaaccaggacaatctcctgaactactgatttactcggcatcctaccggtacactggagtccctgatcgcttcactggcagtggatctgggacggatttcactttcaccatcagcagtgtgcaggctgaagacctggcagtttattactgtcagcatcattatagtactccgtacacgttcggaggggggaccaagctggaaatgaaa

SEQ ID NO: 25 - protein, 447 aa, Artificial Sequence
  Synthetic_7A6 VH3/Vk5-DLE heavy chain
QVQLQESGPGLVKPSQTLSLTCTVTGYSITSDYAWNWIRQPPGKGLEWMGYISYSGSARYNPSLKSRVTISRDTSKNQFSLKLSSVTAEDTATYYCARKGYPAYFAYWGQGTLVTVSSASTKGPSVFPLAPSSKSTSGGTAALGCLVKDYFPEPVTVSWNSGALTSGVHTFPAVLQSSGLYSLSSVVTVPSSSLGTQTYICNVNHKPSNTKVDKRVEPKSCDKTHTCPPCPAPELLGGPDVFLFPPKPKDTLMISRTPEVTCVVVDVSHEDPEVKFNWYVDGVEVHNAKTKPREEQYNSTYRVVSVLTVLHQDWLNGKEYKCKVSNKALPLPEEKTISKAKGQPREPQVYTLPPSREEMTKNQVSLTCLVKGFYPSDIAVEWESNGQPENNYKTTPPVLDSDGSFFLYSKLTVDKSRWQQGNVFSCSVMHEALHNHYTQKSLSLSPG

SEQ ID NO: 26 - protein, 448 aa, Artificial Sequence
  Synthetic_VH3/Vk5 N298A heavy chain
QVQLQESGPGLVKPSQTLSLTCTVTGYSITSDYAWNWIRQPPGKGLEWMGYISYSGSARYNPSLKSRVTISRDTSKNQFSLKLSSVTAEDTATYYCARKGYPAYFAYWGQGTLVTVSSASTKGPSVFPLAPSSKSTSGGTAALGCLVKDYFPEPVTVSWNSGALTSGVHTFPAVLQSSGLYSLSSVVTVPSSSLGTQTYICNVNHKPSNTKVDKRVEPKSCDKTHTCPPCPAPELLGGPSVFLFPPKPKDTLMISRTPEVTCVVVDVSHEDPEVKFNWYVDGVEVHNAKTKPREEQYASTYRVVSVLTVLHQDWLNGKEYKCKVSNKALPAPIEKTISKAKGQPREPQVYTLPPSREEMTKNQVSLTCLVKGFYPSDIAVEWESNGQPENNYKTTPPVLDSDGSFFLYSKLTVDKSRWQQGNVFSCSVMHEALHNHYTQKSLSLSPGK

SEQ ID NO: 27 - protein, 448 aa, Artificial Sequence
  Synthetic_7A6 VH3/Vk5 AAA heavy chain
QVQLQESGPGLVKPSQTLSLTCTVTGYSITSDYAWNWIRQPPGKGLEWMGYISYSGSARYNPSLKSRVTISRDTSKNQFSLKLSSVTAEDTATYYCARKGYPAYFAYWGQGTLVTVSSASTKGPSVFPLAPSSKSTSGGTAALGCLVKDYFPEPVTVSWNSGALTSGVHTFPAVLQSSGLYSLSSVVTVPSSSLGTQTYICNVNHKPSNTKVDKRVEPKSCDKTHTCPPCPAPELLGGPSVFLFPPKPKDTLMISRTPEVTCVVVDVSHEDPEVKFNWYVDGVEVHNAKTKPREEQYNATYRVVSVLTVLHQDWLNGKEYKCKVSNKALPAPIAATISKAKGQPREPQVYTLPPSREEMTKNQVSLTCLVKGFYPSDIAVEWESNGQPENNYKTTPPVLDSDGSFFLYSKLTVDKSRWQQGNVFSCSVMHEALHNHYTQKSLSLSPGK

SEQ ID NO: 28 - protein, 448 aa, Artificial Sequence
  Synthetic_7A6 VH3/Vk5 LALAPG heavy chain
QVQLQESGPGLVKPSQTLSLTCTVTGYSITSDYAWNWIRQPPGKGLEWMGYISYSGSARYNPSLKSRVTISRDTSKNQFSLKLSSVTAEDTATYYCARKGYPAYFAYWGQGTLVTVSSASTKGPSVFPLAPSSKSTSGGTAALGCLVKDYFPEPVTVSWNSGALTSGVHTFPAVLQSSGLYSLSSVVTVPSSSLGTQTYICNVNHKPSNTKVDKRVEPKSCDKTHTCPPCPAPEAAGGPSVFLFPPKPKDTLMISRTPEVTCVVVDVSHEDPEVKFNWYVDGVEVHNAKTKPREEQYNSTYRVVSVLTVLHQDWLNGKEYKCKVSNKALGAPIEKTISKAKGQPREPQVYTLPPSREEMTKNQVSLTCLVKGFYPSDIAVEWESNGQPENNYKTTPPVLDSDGSFFLYSKLTVDKSRWQQGNVFSCSVMHEALHNHYTQKSLSLSPGK

SEQ ID NO: 29 - protein, 214 aa, Artificial Sequence
  Synthetic_Light chain of 7A6 VH3/Vk5 mutants
DIQMTQSPSSLSASVGDRVSITCKASQDVSTAVAWYQQKPGQAPRLLIYSASYRYTGVPDRFSGSGSGTDFTLTISSLQPEDFATYYCQHHYSTPYTFGQGTKLEIKRTVAAPSVFIFPPSDEQLKSGTASVVCLLNNFYPREAKVQWKVDNALQSGNSQESVTEQDSKDSTYSLSSTLTLSKADYEKHKVYACEVTHQGLSSPVTKSFNRGEC

SEQ ID NO: 30 - protein, 244 aa, Artificial Sequence
  Synthetic_human TIGIT
MRWCLLLIWAQGLRQAPLASGMMTGTIETTGNISAEKGGSIILQCHLSSTTAQVTQVNWEQQDQLLAICNADLGWHISPSFKDRVAPGPGLGLTLQSLTVNDTGEYFCIYHTYPDGTYTGRIFLEVLESSVAEHGARFQIPLLGAMAATLVVICTAVIVVVALTRKKKALRIHSVEGDLRRKSAGQEEWSPSAPSPPGSCVQAEAAPAGLCGEQRGEDCAELHDYFNVLSYRSLGNCSFFTETG

SEQ ID NO: 31 - protein, 20 aa, Artificial Sequence
  Synthetic_Epitope region on human TIGIT
TAQVTQVNWEQQDQLLAICN